European Patent Application EP 4 512 416 A2, published February 26, 2025. Title: MUTATIONS IN CANINE ANTIBODY CONSTANT REGIONS. Applicant: Zoetis Services LLC. The sequence listing filed with the application follows.

SEQUENCE LISTING (35 sequences)

SEQ ID NO: 1 - protein, 331 aa, Canis familiaris
  REGION 1..331: note = MISC_FEATURE - The Wildtype Canine IgGA Constant Region
ASTTAPSVFPLAPSCGSTSGSTVALACLVSGYFPEPVTVSWNSGSLTSGVHTFPSVLQSSGLHSLSSMVTVPSSRWPSETFTCNVVHPASNTKVDKPVFNECRCTDTPPCPVPEPLGGPSVLIFPPKPKDILRITRTPEVTCVVLDLGREDPEVQISWFVDGKEVHTAKTQSREQQFNGTYRVVSVLPIEHQDWLTGKEFKCRVNHIDLPSPIERTISKARGRAHKPSVYVLPPSPKELSSSDTVSITCLIKDFYPPDIDVEWQSNGQQEPERKHRMTPPQLDEDGSYFLYSKLSVDKSRWQQGDPFTCAVMHETLQNHYTDLSLSHSPGK

SEQ ID NO: 2 - protein, 335 aa, Canis familiaris
  REGION 1..335: note = MISC_FEATURE - The Wildtype Canine IgGB Constant Region
ASTTAPSVFPLAPSCGSTSGSTVALACLVSGYFPEPVTVSWNSGSLTSGVHTFPSVLQSSGLYSLSSMVTVPSSRWPSETFTCNVAHPASKTKVDKPVPKRENGRVPRPPDCPKCPAPEMLGGPSVFIFPPKPKDTLLIARTPEVTCVVVDLDPEDPEVQISWFVDGKQMQTAKTQPREEQFNGTYRVVSVLPIGHQDWLKGKQFTCKVNNKALPSPIERTISKARGQAHQPSVYVLPPSREELSKNTVSLTCLIKDFFPPDIDVEWQSNGQQEPESKYRTTPPQLDEDGSYFLYSKLSVDKSRWQRGDTFICAVMHEALHNHYTQESLSHSPGK

SEQ ID NO: 3 - protein, 333 aa, Canis familiaris
  REGION 1..333: note = MISC_FEATURE - The Wildtype Canine IgGC Constant Region
ASTTAPSVFPLAPSCGSQSGSTVALACLVSGYIPEPVTVSWNSVSLTSGVHTFPSVLQSSGLYSLSSMVTVPSSRWPSETFTCNVAHPATNTKVDKPVAKECECKCNCNNCPCPGCGLLGGPSVFIFPPKPKDILVTARTPTVTCVVVDLDPENPEVQISWFVDSKQVQTANTQPREEQSNGTYRVVSVLPIGHQDWLSGKQFKCKVNNKALPSPIEEIISKTPGQAHQPNVYVLPPSRDEMSKNTVTLTCLVKDFFPPEIDVEWQSNGQQEPESKYRMTPPQLDEDGSYFLYSKLSVDKSRWQRGDTFICAVMHEALHNHYTQISLSHSPGK

SEQ ID NO: 4 - protein, 331 aa, Canis familiaris
  REGION 1..331: note = MISC_FEATURE - The Wildtype Canine IgGD Constant Region
ASTTAPSVFPLAPSCGSTSGSTVALACLVSGYFPEPVTVSWNSGSLTSGVHTFPSVLQSSGLYSLSSTVTVPSSRWPSETFTCNVVHPASNTKVDKPVPKESTCKCISPCPVPESLGGPSVFIFPPKPKDILRITRTPEITCVVLDLGREDPEVQISWFVDGKEVHTAKTQPREQQFNSTYRVVSVLPIEHQDWLTGKEFKCRVNHIGLPSPIERTISKARGQAHQPSVYVLPPSPKELSSSDTVTLTCLIKDFFPPEIDVEWQSNGQPEPESKYHTTAPQLDEDGSYFLYSKLSVDKSRWQQGDTFTCAVMHEALQNHYTDLSLSHSPGK

SEQ ID NO: 5 - DNA, 1005 bp, Canis familiaris
  misc_feature 1..1005: note = The Wildtype Canine IgGB constant domain - codon optimized.
  source 1..1005: mol_type = genomic DNA
gccagcaccacagctccctccgtgttccccctggctcctagctgcggctctacctccggcagcacagtggccctggcttgtctggtgtccggctacttccctgagccagtgaccgtgagctggaactccggctccctgacctccggagtgcacacatttccaagcgtgctgcagtcttccggcctgtattctctgagctctatggtgaccgtgccttccagcaggtggccatctgagacattcacctgcaacgtggcccatcccgcttccaagacaaaggtggacaagcccgtgcctaagagggagaatggaagggtgccccggccccctgattgccctaagtgtccagctccagagatgctgggaggaccatccgtgttcatctttccacccaagcccaaggataccctgctgatcgctagaacccctgaggtgacatgcgtggtggtggacctggatccagaggaccccgaggtgcagatctcttggttcgtggatggcaagcagatgcagaccgccaagacacagcctagggaggagcagtttaacggcacctacagggtggtgtccgtgctgccaatcggccaccaggactggctgaagggcaagcagtttacctgcaaggtgaacaataaggctctgccttctccaatcgagagaacaatctccaaggccaggggccaggctcatcagcctagcgtgtacgtgctgcctccatccagagaggagctgagcaagaacaccgtgtctctgacatgtctgatcaaggatttctttccccctgacatcgatgtggagtggcagagcaatggccagcaggagccagagtctaagtatcgcaccacaccaccccagctggacgaggatggcagctacttcctgtatagcaagctgtctgtggacaagtctagatggcagcgcggcgatacctttatctgtgccgtgatgcacgaggcactgcacaatcactacacccaggagagtctgagccacagcccaggaaaa

SEQ ID NO: 6 - DNA, 1005 bp, Canis familiaris
  misc_feature 1..1005: note = The wildtype canine IgGB constant domain
  source 1..1005: mol_type = genomic DNA
gcctcaacaactgctcctagcgtgtttcccctggcccctagctgcggaagtacctcaggcagcacagtggccctggcttgtctggtgtctggatatttccctgagccagtgaccgtgagttggaacagcggctctctgacctccggggtgcacacatttccatctgtgctgcagtctagtggcctgtactccctgtcaagcatggtgactgtgccttcctctaggtggccatcagaaactttcacctgcaacgtggcccatcccgccagcaagaccaaagtggacaagcccgtgcctaaaagggagaatggaagggtgccaagaccacctgattgccctaagtgtccagctccagaaatgctgggaggaccaagcgtgttcatctttccacccaagcccaaagacacactgctgattgctagaactcccgaggtgacctgcgtggtggtggacctggatccagaggaccccgaagtgcagatctcctggttcgtggatgggaagcagatgcagacagccaaaactcagcctcgggaggaacagtttaacggaacctatagagtggtgtctgtgctgccaattggacaccaggactggctgaagggcaaacagtttacatgcaaggtgaacaacaaggccctgcctagtccaatcgagaggactatttcaaaagctaggggacaggctcatcagccttccgtgtatgtgctgcctccatcccgggaggaactgtctaagaacacagtgagtctgacttgtctgatcaaagatttctttccccctgacattgatgtggagtggcagagcaatgggcagcaggagccagaatccaagtacagaaccacaccaccccagctggacgaagatggctcctatttcctgtacagtaagctgtcagtggacaaatctaggtggcagcgcggggatacctttatctgcgccgtgatgcacgaggctctgcacaatcattacacacaagaaagtctgtcacatagccccggcaag

SEQ ID NO: 7 - protein, 98 aa, Canis familiaris
  REGION 1..98: note = MISC_FEATURE - The wildtype canine IgGB CH1 Domain
ASTTAPSVFPLAPSCGSTSGSTVALACLVSGYFPEPVTVSWNSGSLTSGVHTFPSVLQSSGLYSLSSMVTVPSSRWPSETFTCNVAHPASKTKVDKPV

SEQ ID NO: 8 - protein, 18 aa, Canis familiaris
  REGION 1..18: note = MISC_FEATURE - The wildtype canine IgGB Hinge Domain
PKRENGRVPRPPDCPKCP

SEQ ID NO: 9 - protein, 110 aa, Canis familiaris
  REGION 1..110: note = MISC_FEATURE - The wildtype canine IgGB CH2 Domain
APEMLGGPSVFIFPPKPKDTLLIARTPEVTCVVVDLDPEDPEVQISWFVDGKQMQTAKTQPREEQFNGTYRVVSVLPIGHQDWLKGKQFTCKVNNKALPSPIERTISKAR

SEQ ID NO: 10 - protein, 109 aa, Canis familiaris
  REGION 1..109: note = MISC_FEATURE - The wildtype canine IgGB CH3 Domain
GQAHQPSVYVLPPSREELSKNTVSLTCLIKDFFPPDIDVEWQSNGQQEPESKYRTTPPQLDEDGSYFLYSKLSVDKSRWQRGDTFICAVMHEALHNHYTQESLSHSPGK

SEQ ID NO: 11 - DNA, 294 bp, Canis familiaris
  misc_feature 1..294: note = The wildtype canine IgGB CH1 Domain
  source 1..294: mol_type = genomic DNA
gcctcaacaactgctcctagcgtgtttcccctggcccctagctgcggaagtacctcaggcagcacagtggccctggcttgtctggtgtctggatatttccctgagccagtgaccgtgagttggaacagcggctctctgacctccggggtgcacacatttccatctgtgctgcagtctagtggcctgtactccctgtcaagcatggtgactgtgccttcctctaggtggccatcagaaactttcacctgcaacgtggcccatcccgccagcaagaccaaagtggacaagcccgtg

SEQ ID NO: 12 - DNA, 54 bp, Canis familiaris
  misc_feature 1..54: note = The wildtype canine IgGB Hinge Domain
  source 1..54: mol_type = genomic DNA
cctaaaagggagaatggaagggtgccaagaccacctgattgccctaagtgtcca

SEQ ID NO: 13 - DNA, 330 bp, Canis familiaris
  misc_feature 1..330: note = The wildtype canine IgGB CH2 Domain
  source 1..330: mol_type = genomic DNA
gctccagaaatgctgggaggaccaagcgtgttcatctttccacccaagcccaaagacacactgctgattgctagaactcccgaggtgacctgcgtggtggtggacctggatccagaggaccccgaagtgcagatctcctggttcgtggatgggaagcagatgcagacagccaaaactcagcctcgggaggaacagtttaacggaacctatagagtggtgtctgtgctgccaattggacaccaggactggctgaagggcaaacagtttacatgcaaggtgaacaacaaggccctgcctagtccaatcgagaggactatttcaaaagctagg

SEQ ID NO: 14 - DNA, 327 bp, Canis familiaris
  misc_feature 1..327: note = The wildtype canine IgGB CH3 Domain
  source 1..327: mol_type = genomic DNA
ggacaggctcatcagccttccgtgtatgtgctgcctccatcccgggaggaactgtctaagaacacagtgagtctgacttgtctgatcaaagatttctttccccctgacattgatgtggagtggcagagcaatgggcagcaggagccagaatccaagtacagaaccacaccaccccagctggacgaagatggctcctatttcctgtacagtaagctgtcagtggacaaatctaggtggcagcgcggggatacctttatctgcgccgtgatgcacgaggctctgcacaatcattacacacaagaaagtctgtcacatagccccggcaag

SEQ ID NO: 15 - protein, 330 aa, Homo sapiens [sequence omitted]

SEQ ID NO: 16 - DNA, 993 bp, Canis familiaris
  misc_feature 1..993: note = The Wildtype Canine IgGA Constant Region
  source 1..993: mol_type = genomic DNA
gcctccaccacggcgccctcggttttcccactggcccccagctgcgggtccacttccggctccacggtggccctggcctgcctggtgtcaggctacttccccgagcctgtaactgtgtcctggaactccggctccttgaccagcggtgtgcacaccttcccgtccgtcctgcagtcctcagggcttcactccctcagcagcatggtgacagtgccctccagcaggtggcccagcgagaccttcacctgcaacgtggtccacccagccagcaacactaaagtagacaagccagtgttcaatgaatgcagatgcactgatacacccccatgcccagtccctgaacctctgggagggccttcggtcctcatctttcccccgaaacccaaggacatcctcaggattacccgaacacccgaggtcacctgtgtggtgttagatctgggccgtgaggaccctgaggtgcagatcagctggttcgtggatggtaaggaggtgcacacagccaagacccagtctcgtgagcagcagttcaacggcacctaccgtgtggtcagcgtcctccccattgagcaccaggactggctcacagggaaggagttcaagtgcagagtcaaccacatagacctcccgtctcccatcgagaggaccatctctaaggccagagggagggcccataagcccagtgtgtatgtcctgccgccatccccaaaggagttgtcatccagtgacacagtcagcatcacctgcctgataaaagacttctacccacctgacattgatgtggagtggcagagcaatggacagcaggagcccgagaggaagcaccgcatgaccccgccccagctggacgaggacgggtcctacttcctgtacagcaagctctctgtggacaagagccgctggcagcagggagaccccttcacatgtgcggtgatgcatgaaactctacagaaccactacacagatctatccctctcccattctccgggtaaa

SEQ ID NO: 17 - DNA, 999 bp, Canis familiaris
  misc_feature 1..999: note = The Wildtype Canine IgGC Constant Region
  source 1..999: mol_type = genomic DNA
gcctccaccacggcgccctcggttttcccactggcccccagctgtgggtcccaatccggctccacggtggccctggcctgcctggtgtcaggctacatccccgagcctgtaactgtgtcctggaactccgtctccttgaccagcggtgtgcacaccttcccgtccgtcctgcagtcctcagggctctactccctcagcagcatggtgacagtgccctccagcaggtggcccagcgagaccttcacctgcaatgtggcccacccggccaccaacactaaagtagacaagccagtggccaaagaatgcgagtgcaagtgtaactgtaacaactgcccatgcccaggttgtggcctgctgggagggccttcggtcttcatctttcccccaaaacccaaggacatcctcgtgactgcccggacacccacagtcacttgtgtggtggtggatctggacccagaaaaccctgaggtgcagatcagctggttcgtggatagtaagcaggtgcaaacagccaacacgcagcctcgtgaggagcagtccaatggcacctaccgtgtggtcagtgtcctccccattgggcaccaggactggctttcagggaagcagttcaagtgcaaagtcaacaacaaagccctcccatcccccattgaggagatcatctccaagaccccagggcaggcccatcagcctaatgtgtatgtcctgccgccatcgcgggatgagatgagcaagaatacggtcaccctgacctgtctggtcaaagacttcttcccacctgagattgatgtggagtggcagagcaatggacagcaggagcctgagagcaagtaccgcatgaccccgccccagctggatgaagatgggtcctacttcctatacagcaagctctccgtggacaagagccgctggcagcggggagacaccttcatatgtgcggtgatgcatgaagctctacacaaccactacacacagatatccctctcccattctccgggtaaa

SEQ ID NO: 18 - DNA, 993 bp, Canis familiaris
  misc_feature 1..993: note = The Wildtype Canine IgGD Constant Region
  source 1..993: mol_type = genomic DNA
gcctccaccacggcgccctcggttttcccactggcccccagctgcgggtccacttccggctccacggtggccctggcctgcctggtgtcaggctacttccccgagcctgtaactgtgtcctggaactccggctccttgaccagcggtgtgcacaccttcccgtccgtcctgcagtcctcagggctctactccctcagcagcacggtgacagtgccctccagcaggtggcccagcgagaccttcacctgcaacgtggtccacccggccagcaacactaaagtagacaagccagtgcccaaagagtccacctgcaagtgtatatccccatgcccagtccctgaatcactgggagggccttcggtcttcatctttcccccgaaacccaaggacatcctcaggattacccgaacacccgagatcacctgtgtggtgttagatctgggccgtgaggaccctgaggtgcagatcagctggttcgtggatggtaaggaggtgcacacagccaagacgcagcctcgtgagcagcagttcaacagcacctaccgtgtggtcagcgtcctccccattgagcaccaggactggctcaccggaaaggagttcaagtgcagagtcaaccacataggcctcccgtcccccatcgagaggactatctccaaagccagagggcaagcccatcagcccagtgtgtatgtcctgccaccatccccaaaggagttgtcatccagtgacacggtcaccctgacctgcctgatcaaagacttcttcccacctgagattgatgtggagtggcagagcaatggacagccggagcccgagagcaagtaccacacgactgcgccccagctggacgaggacgggtcctacttcctgtacagcaagctctctgtggacaagagccgctggcagcagggagacaccttcacatgtgcggtgatgcatgaagctctacagaaccactacacagatctatccctctcccattctccgggtaaa

SEQ ID NO: 19 - DNA, 990 bp, Homo sapiens
  misc_feature 1..990: note = The Wildtype Human IgG1 Constant Region
  source 1..990: mol_type = genomic DNA
gcctccaccaagggcccatcggtcttccccctggcaccctcctccaagagcacctctgggggcacagcggccctgggctgcctggtcaaggactacttccccgaaccggtgacggtgtcgtggaactcaggcgccctgaccagcggcgtgcacaccttcccggctgtcctacagtcctcaggactctactccctcagcagcgtggtgaccgtgccctccagcagcttgggcacccagacctacatctgcaacgtgaatcacaagcccagcaacaccaaggtggacaagaaagttgagcccaaatcttgtgacaaaactcacacatgcccaccgtgcccagcacctgaactcctggggggaccgtcagtcttcctcttccccccaaaacccaaggacaccctcatgatctcccggacccctgaggtcacatgcgtggtggtggacgtgagccacgaagaccctgaggtcaagttcaactggtacgtggacggcgtggaggtgcataatgccaagacaaagccgcgggaggagcagtacaacagcacgtaccgtgtggtcagcgtcctcaccgtcctgcaccaggactggctgaatggcaaggagtacaagtgcaaggtctccaacaaagccctcccagcccccatcgagaaaaccatctccaaagccaaagggcagccccgagaaccacaggtgtacaccctgcccccatcccgggatgagctgaccaagaaccaggtcagcctgacctgcctggtcaaaggcttctatcccagcgacatcgccgtggagtgggagagcaatgggcagccggagaacaactacaagaccacgcctcccgtgctggactccgacggctccttcttcctctacagcaagctcaccgtggacaagagcaggtggcagcaggggaacgtcttctcatgctccgtgatgcatgaggctctgcacaaccactacacgcagaagagcctctccctgtctccgggtaaa

SEQ ID NO: 20 - DNA, 15 bp, Mus musculus
  misc_feature 1..15: note = Heavy Chain CDR1
  source 1..15: mol_type = genomic DNA
aactacggcatgagc

SEQ ID NO: 21 - protein, 5 aa, Mus musculus
  REGION 1..5: note = MISC_FEATURE - Heavy Chain CDR1
NYGMS

SEQ ID NO: 22 - DNA, 51 bp, Mus musculus
  misc_feature 1..51: note = Heavy Chain CDR2
  source 1..51: mol_type = genomic DNA
accatcagctacggcggcagctacacctactaccccgacaacatcaagggc

SEQ ID NO: 23 - protein, 17 aa, Mus musculus
  REGION 1..17: note = MISC_FEATURE - Heavy Chain CDR2
TISYGGSYTYYPDNIKG

SEQ ID NO: 24 - DNA, 33 bp, Mus musculus
  misc_feature 1..33: note = Heavy Chain CDR3
  source 1..33: mol_type = genomic DNA
gtgcggggctacggctacgacacaatggactac

SEQ ID NO: 25 - protein, 11 aa, Mus musculus
  REGION 1..11: note = MISC_FEATURE - Heavy Chain CDR3
VRGYGYDTMDY

SEQ ID NO: 26 - DNA, 45 bp, Mus musculus
  misc_feature 1..45: note = Light Chain CDR1
  source 1..45: mol_type = genomic DNA
aaggccagccagagcgtgtccttcgccggcacaggcctgatgcac

SEQ ID NO: 27 - protein, 15 aa, Mus musculus
  REGION 1..15: note = MISC_FEATURE - Light Chain CDR1
KASQSVSFAGTGLMH

SEQ ID NO: 28 - DNA, 21 bp, Mus musculus
  misc_feature 1..21: note = Light Chain CDR2
  source 1..21: mol_type = genomic DNA
cgggccagcaacctggaagcc

SEQ ID NO: 29 - protein, 7 aa, Mus musculus
  REGION 1..7: note = MISC_FEATURE - Light Chain CDR2
RASNLEA

SEQ ID NO: 30 - DNA, 27 bp, Mus musculus
  misc_feature 1..27: note = Light Chain CDR3
  source 1..27: mol_type = genomic DNA
cagcagagcagagagtacccctggacc

SEQ ID NO: 31 - protein, 9 aa, Mus musculus
  REGION 1..9: note = MISC_FEATURE - Light Chain CDR3
QQSREYPWT

SEQ ID NO: 32 - DNA, 657 bp, synthetic construct
  misc_feature 1..657: note = ZTS-8183 - Variable Light Nucleic Acid Sequence - Caninized
  source 1..657: mol_type = other DNA
gagatcgtgatgacccagagccccgccagcctgagcctgagccaggaagagaaagtcaccatcacatgcaaggccagccagagcgtgtccttcgccggcacaggcctgatgcactggtatcagcagaagcccggccaggcccccaagctgctgatctaccgggccagcaacctggaagccggcgtgccaagcagattcagcggcagcggctccggcaccgacttcagcttcaccatcagcagcctcgaacccgaggacgtggccgtgtactactgccagcagagcagagagtacccctggaccttcggccagggtaccaagctggaaatcaagcggaacgacgcccagcccgccgtgtacctgttccagcccagccccgatcagctgcacaccggcagcgcttcagtcgtctgcctgctgaacagcttctaccccaaggacatcaacgtgaagtggaaggtggacggcgtgatccaggacaccggcatccaggaaagcgtcaccgagcaggacaaggacagcacctacagcctgagcagcaccctgaccatgtccagcaccgagtacctgagccacgagctgtatagctgcgagatcacccacaagagcctgcctagcaccctgatcaagagcttccagcggagcgagtgctagtag

SEQ ID NO: 33 - protein, 217 aa, synthetic construct
  REGION 1..217: note = ZTS-8183 - Variable Light Amino Acid Sequence - Caninized
EIVMTQSPASLSLSQEEKVTITCKASQSVSFAGTGLMHWYQQKPGQAPKLLIYRASNLEAGVPSRFSGSGSGTDFSFTISSLEPEDVAVYYCQQSREYPWTFGQGTKLEIKRNDAQPAVYLFQPSPDQLHTGSASVVCLLNSFYPKDINVKWKVDGVIQDTGIQESVTEQDKDSTYSLSSTLTMSSTEYLSHELYSCEITHKSLPSTLIKSFQRSEC

SEQ ID NO: 34 - DNA, 1365 bp, synthetic construct
  misc_feature 1..1365: note = ZTS-8183 - Variable Heavy Nucleic Acid Sequence - Caninized
  source 1..1365: mol_type = other DNA
gaggtgcagctggtggaatctggcggcgacctggtcaagcctggcggcagcctgagactgagctgtgtggccagcggcttcaccttcagcaactacggcatgagctgggtccgacaggcccctggcaagggactgcagtgggtggccaccatcagctacggcggcagctacacctactaccccgacaacatcaagggccggttcaccatcagccgggacaacgccaagaacaccctgtacctgcagatgaacagcctgcgggccgaggacaccgccatgtactactgcgtgcggggctacggctacgacacaatggactactggggccagggcaccctcgtgaccgtctcgagcgcctcaacaactgctcctagcgtgtttcccctggcccctagctgcggaagtacctcaggcagcacagtggccctggcttgtctggtgtctggatatttccctgagccagtgaccgtgagttggaacagcggctctctgacctccggggtgcacacatttccatctgtgctgcagtctagtggcctgtactccctgtcaagcatggtgactgtgccttcctctaggtggccatcagaaactttcacctgcaacgtggcccatcccgccagcaagaccaaagtggacaagcccgtgcctaaaagggagaatggaagggtgccaagaccacctgattgccctaagtgtccagctccagaaatgctgggaggaccaagcgtgttcatctttccacccaagcccaaagacacactgctgattgctagaactcccgaggtgacctgcgtggtggtggacctggatccagaggaccccgaagtgcagatctcctggttcgtggatgggaagcagatgcagacagccaaaactcagcctcgggaggaacagtttaacggaacctatagagtggtgtctgtgctgccaattggacaccaggactggctgaagggcaaacagtttacatgcaaggtgaacaacaaggccctgcctagtccaatcgagaggactatttcaaaagctaggggacaggctcatcagccttccgtgtatgtgctgcctccatcccgggaggaactgtctaagaacacagtgagtctgacttgtctgatcaaagatttctttccccctgacattgatgtggagtggcagagcaatgggcagcaggagccagaatccaagtacagaaccacaccaccccagctggacgaagatggctcctatttcctgtacagtaagctgtcagtggacaaatctaggtggcagcgcggggatacctttatctgcgccgtgatgcacgaggctctgcaccatcattacacacaagaaagtctgtcacatagccccggcaagtagtag

SEQ ID NO: 35 - protein, 453 aa, synthetic construct
  REGION 1..453: note = ZTS-8183 - Variable Heavy Amino Acid Sequence - Caninized
EVQLVESGGDLVKPGGSLRLSCVASGFTFSNYGMSWVRQAPGKGLQWVATISYGGSYTYYPDNIKGRFTISRDNAKNTLYLQMNSLRAEDTAMYYCVRGYGYDTMDYWGQGTLVTVSSASTTAPSVFPLAPSCGSTSGSTVALACLVSGYFPEPVTVSWNSGSLTSGVHTFPSVLQSSGLYSLSSMVTVPSSRWPSETFTCNVAHPASKTKVDKPVPKRENGRVPRPPDCPKCPAPEMLGGPSVFIFPPKPKDTLLIARTPEVTCVVVDLDPEDPEVQISWFVDGKQMQTAKTQPREEQFNGTYRVVSVLPIGHQDWLKGKQFTCKVNNKALPSPIERTISKARGQAHQPSVYVLPPSREELSKNTVSLTCLIKDFFPPDIDVEWQSNGQQEPESKYRTTPPQLDEDGSYFLYSKLSVDKSRWQRGDTFICAVMHEALHHHYTQESLSHSPGK